European Patent Application EP 4 180 451 A1, published May 17, 2023. Title: GLP-1/GLUCAGON DUAL AGONIST FUSION PROTEIN. Applicant: DONGGUAN YUNJING BIOTECHNOLOGY CO., LTD. The sequence listing filed with the application follows.

SEQUENCE LISTING (14 sequences)

SEQ ID NO: 1 - protein, 39 aa, Artificial Sequence
  Peptide Design Template
  MISC_FEATURE (2)..(2): X = Gly or Ser
  MISC_FEATURE (10)..(10): X = Leu or Tyr
  MISC_FEATURE (18)..(18): X = Arg or Ala
  MISC_FEATURE (20)..(20): X = Lys or Gln
  MISC_FEATURE (21)..(21): X = Glu or Asp
  MISC_FEATURE (23)..(23): X = Ile or Val
  MISC_FEATURE (24)..(24): X = Ala or Gln
HXQGTFTSDXSKYLDEQXAXXFXXWLIAGGPSSGAPPPS

SEQ ID NO: 2 - protein, 19 aa, Artificial Sequence
  Signal Peptide
MELGLRWVFLVAILEGVQC

SEQ ID NO: 3 - protein, 39 aa, Artificial Sequence
  GLP-1/Glucagon Dual Agonist
HGQGTFTSDLSKYLDEQRAKEFIAWLIAGGPSSGAPPPS

SEQ ID NO: 4 - DNA, 174 bp, Artificial Sequence
  Nucleotide Sequence Encoding Signal Peptide and GLP-1/Glucagon Dual Agonist
atggagctgggcctgaggtgggtgttcctggtggccatcctggagggcgtgcagtgccacggccagggcaccttcaccagcgacctgagcaagtacctggacgagcagagggccaaggagttcatcgcctggctgatcgccggcggccccagcagcggcgcccccccccccagc

SEQ ID NO: 5 - DNA, 33 bp, Artificial Sequence
  Primer
gacgagcagrsggccmaggasttcrthsmctgg

SEQ ID NO: 6 - DNA, 42 bp, Artificial Sequence
  Primer
caggtacttgctawrgtcgctggtgaaggtgccctgtysgtg

SEQ ID NO: 7 - protein, 39 aa, Artificial Sequence
  3D9
HSQGTFTSDYSKYLDEQAAKEFIAWLIAGGPSSGAPPPS

SEQ ID NO: 8 - protein, 39 aa, Artificial Sequence
  6B7
HSQGTFTSDYSKYLDEQRAKDFIAWLIAGGPSSGAPPPS

SEQ ID NO: 9 - protein, 39 aa, Artificial Sequence
  12C6
HSQGTFTSDYSKYLDEQRAKEFVAWLIAGGPSSGAPPPS

SEQ ID NO: 10 - protein, 17 aa, Artificial Sequence
  Linker Sequence
GGGGGSGGGGSGGGGSA

SEQ ID NO: 11 - protein, 228 aa, Homo sapiens
ESKYGPPCPPCPAPEAAGGPSVFLFPPKPKDTLMISRTPEVTCVVVDVSQEDPEVQFNWYVDGVEVHNAKTKPREEQFNSTYRVVSVLTVLHQDWLNGKEYKCKVSNKGLPSSIEKTISKAKGQPREPQVYTLPPSQEEMTKNQVSLTCLVKGFYPSDIAVEWESNGQPENNYKTTPPVLDSDGSFFLYSRLTVDKSRWQEGNVFSCSVMHEALHNHYTQKSLSLSLG

SEQ ID NO: 12 - protein, 284 aa, Artificial Sequence
  Fc Fusion Protein 1
HSQGTFTSDYSKYLDEQAAKEFIAWLIAGGPSSGAPPPSGGGGGSGGGGSGGGGSAESKYGPPCPPCPAPEAAGGPSVFLFPPKPKDTLMISRTPEVTCVVVDVSQEDPEVQFNWYVDGVEVHNAKTKPREEQFNSTYRVVSVLTVLHQDWLNGKEYKCKVSNKGLPSSIEKTISKAKGQPREPQVYTLPPSQEEMTKNQVSLTCLVKGFYPSDIAVEWESNGQPENNYKTTPPVLDSDGSFFLYSRLTVDKSRWQEGNVFSCSVMHEALHNHYTQKSLSLSLG

SEQ ID NO: 13 - protein, 284 aa, Artificial Sequence
  Fc Fusion Protein 2
HSQGTFTSDYSKYLDEQRAKDFIAWLIAGGPSSGAPPPSGGGGGSGGGGSGGGGSAESKYGPPCPPCPAPEAAGGPSVFLFPPKPKDTLMISRTPEVTCVVVDVSQEDPEVQFNWYVDGVEVHNAKTKPREEQFNSTYRVVSVLTVLHQDWLNGKEYKCKVSNKGLPSSIEKTISKAKGQPREPQVYTLPPSQEEMTKNQVSLTCLVKGFYPSDIAVEWESNGQPENNYKTTPPVLDSDGSFFLYSRLTVDKSRWQEGNVFSCSVMHEALHNHYTQKSLSLSLG

SEQ ID NO: 14 - protein, 284 aa, Artificial Sequence
  Fc Fusion Protein 3
HSQGTFTSDYSKYLDEQRAKEFVAWLIAGGPSSGAPPPSGGGGGSGGGGSGGGGSAESKYGPPCPPCPAPEAAGGPSVFLFPPKPKDTLMISRTPEVTCVVVDVSQEDPEVQFNWYVDGVEVHNAKTKPREEQFNSTYRVVSVLTVLHQDWLNGKEYKCKVSNKGLPSSIEKTISKAKGQPREPQVYTLPPSQEEMTKNQVSLTCLVKGFYPSDIAVEWESNGQPENNYKTTPPVLDSDGSFFLYSRLTVDKSRWQEGNVFSCSVMHEALHNHYTQKSLSLSLG